European Patent Application EP 4 349 358 A1, published April 10, 2024. Title: Inhibitor of transmembrane 4 L6 family member 19 and novel uses thereof. Applicant: MedPacto Inc. The sequence listing filed with the application follows.

SEQUENCE LISTING (21 sequences)

SEQ ID NO: 1 - protein, 209 aa, Homo sapiens
MVSSPCTQASSRTCSRILGLSLGTAALFAAGANVALLLPNWDVTYLLRGLLGRHAMLGTGLWGGGLMVLTAAILISLMGWRYGCFSKSGLCRSVLTALLSGGLALLGALICFVTSGVALKDGPFCMFDVSSFNQTQAWKYGYPFKDLHSRNYLYDRSLWNSVCLEPSAAVVWHVSLFSALLCISLLQLLLVVVHVINSLLGLFCSLCEK

SEQ ID NO: 2 - protein, 242 aa, Homo sapiens
MVSSPCTQASSRTCSRILGLSLGTAALFAAGANVALLLPNWDVTYLLRGLLGRHAMLGTGLWGGGLMVLTAAILISLMGWRYGCFSKSGLCRSVLTALLSGGLALLGALICFVTSGVALKDGPFCMFDVSSFNQTQAWKYGYPFKDLHRIICMTVRSGTPSAWSPLQLLSGTCPSSPPFCASACSSFSWWSFMSSTASWAFSAASARSDRQNLHLQAWVFSSSAVLNPFYKEWVRIINKLPL

SEQ ID NO: 3 - protein, 183 aa, Homo sapiens
MVSSPCTQASSRTCSRILGLSLGTAALFAAGANVALLLPNWDVTYLLRGLLGRHAMLGTGLWGGGLMVLTALLSGGLALLGALICFVTSGVALKDGPFCMFDVSSFNQTQAWKYGYPFKDLHSRNYLYDRSLWNSVCLEPSAAVVWHVSLFSALLCISLLQLLLVVVHVINSLLGLFCSLCEK

SEQ ID NO: 4 - DNA, 1026 bp, Homo sapiens
aaagagtcctggaaagacaaccttcaggtccagccctggagctggaggagtggagccccactctgaagacgcagcctttctccaggttctgtctctcccattctgattcttgacaccagatgcaggatggtgtcctctccctgcacgcaggcaagctcacggacttgctcccgtatcctgggactgagccttgggactgcagccctgtttgctgctggggccaacgtggcactcctccttcctaactgggatgtcacctacctgttgaggggcctccttggcaggcatgccatgctgggaactgggctctggggaggaggcctcatggtactcactgcagctatcctcatctccttgatgggctggagatacggctgcttcagtaagagtgggctctgtcgaagcgtgcttactgctctgttgtcaggtggcctggctttacttggagccctgatttgctttgtcacttctggagttgctctgaaagatggtcctttttgcatgtttgatgtttcatccttcaatcagacacaagcttggaaatatggttacccattcaaagacctgcatagtaggaattatctgtatgaccgttcgctctggaactccgtctgcctggagccctctgcagctgttgtctggcacgtgtccctcttctccgcccttctgtgcatcagcctgctccagcttctcctggtggtcgttcatgtcatcaacagcctcctgggccttttctgcagcctctgcgagaagtgacaggcagaaccttcacttgcaagcatgggtgttttcatcatcggctgtcttgaatcctttctacaaggagtgggtacgaattataaacaaacttcccctttaggtatccctggagtaataatgacaacaaaattcactgcaggtcggtggaatgatagaatgcattttaaatcacattgtaaacttccaggtgatccatggataggataaataactaagttattataattgtttaggaatttatagtccataaaatatcctccagccagg

SEQ ID NO: 5 - DNA, 1022 bp, Homo sapiens
aaagagtcctggaaagacaaccttcaggtccagccctggagctggaggagtggagccccactctgaagacgcagcctttctccaggttctgtctctcccattctgattcttgacaccagatgcaggatggtgtcctctccctgcacgcaggcaagctcacggacttgctcccgtatcctgggactgagccttgggactgcagccctgtttgctgctggggccaacgtggcactcctccttcctaactgggatgtcacctacctgttgaggggcctccttggcaggcatgccatgctgggaactgggctctggggaggaggcctcatggtactcactgcagctatcctcatctccttgatgggctggagatacggctgcttcagtaagagtgggctctgtcgaagcgtgcttactgctctgttgtcaggtggcctggctttacttggagccctgatttgctttgtcacttctggagttgctctgaaagatggtcctttttgcatgtttgatgtttcatccttcaatcagacacaagcttggaaatatggttacccattcaaagacctgcatagaattatctgtatgaccgttcgctctggaactccgtctgcctggagccctctgcagctgttgtctggcacgtgtccctcttctccgcccttctgtgcatcagcctgctccagcttctcctggtggtcgttcatgtcatcaacagcctcctgggccttttctgcagcctctgcgagaagtgacaggcagaaccttcacttgcaagcatgggtgttttcatcatcggctgtcttgaatcctttctacaaggagtgggtacgaattataaacaaacttcccctttaggtatccctggagtaataatgacaacaaaattcactgcaggtcggtggaatgatagaatgcattttaaatcacattgtaaacttccaggtgatccatggataggataaataactaagttattataattgtttaggaatttatagtccataaaatatcctccagccagg

SEQ ID NO: 6 - DNA, 948 bp, Homo sapiens
aaagagtcctggaaagacaaccttcaggtccagccctggagctggaggagtggagccccactctgaagacgcagcctttctccaggttctgtctctcccattctgattcttgacaccagatgcaggatggtgtcctctccctgcacgcaggcaagctcacggacttgctcccgtatcctgggactgagccttgggactgcagccctgtttgctgctggggccaacgtggcactcctccttcctaactgggatgtcacctacctgttgaggggcctccttggcaggcatgccatgctgggaactgggctctggggaggaggcctcatggtgcttactgctctgttgtcaggtggcctggctttacttggagccctgatttgctttgtcacttctggagttgctctgaaagatggtcctttttgcatgtttgatgtttcatccttcaatcagacacaagcttggaaatatggttacccattcaaagacctgcatagtaggaattatctgtatgaccgttcgctctggaactccgtctgcctggagccctctgcagctgttgtctggcacgtgtccctcttctccgcccttctgtgcatcagcctgctccagcttctcctggtggtcgttcatgtcatcaacagcctcctgggccttttctgcagcctctgcgagaagtgacaggcagaaccttcacttgcaagcatgggtgttttcatcatcggctgtcttgaatcctttctacaaggagtgggtacgaattataaacaaacttcccctttaggtatccctggagtaataatgacaacaaaattcactgcaggtcggtggaatgatagaatgcattttaaatcacattgtaaacttccaggtgatccatggataggataaataactaagttattataattgtttaggaatttatagtccataaaatatcctccagccagg

SEQ ID NO: 7 - protein, 206 aa, Mus musculus
MLSFSRVVNCSRTCSRFLGLSLGTASLCAAGANIALLFPNWDVTYLMRGLIGKHAMLGSGLWGGGLMVLLAATLISMTGSFSKSAPCLQVLIALLSSGLALLGAVICFVTSGVALKDGPFCMFDVSSFNQTQAWKFGYPFKDLHNRNYLYDRSLWTSVCLEPSKAVVWHVAFFSILLCISLLQLLLVAIHLVNSILGLFCSFCEKH

SEQ ID NO: 8 - protein, 50 aa, Mus musculus
KDGPFCMFDVSSFNQTQAWKFGYPFKDLHNRNYLYDRSLWTSVCLEPSKA

SEQ ID NO: 9 - protein, 232 aa, Artificial Sequence
  hIgG1-Fc
EPKSCDKTHTCPPCPAPELLGGPSVFLFPPKPKDTLMISRTPEVTCVVVDVSHEDPEVKFNWYVDGVEVHNAKTKPREEQYNSTYRVVSVLTVLHQDWLNGKEYKCKVSNKALPAPIEKTISKAKGQPREPQVYTLPPSRDELTKNQVSLTCLVKGFYPSDIAVEWESNGQPENNYKTTPPVLDSDGSFFLYSKLTVDKSRWQQGNVFSCSVMHEALHNHYTQKSLSLSPGK

SEQ ID NO: 10 - protein, 284 aa, Artificial Sequence
  Mouse TM4SF19(116-165)-Fc fusion protein
KDGPFCMFDVSSFNQTQAWKFGYPFKDLHNRNYLYDRSLWTSVCLEPSKATSEPKSCDKTHTCPPCPAPELLGGPSVFLFPPKPKDTLMISRTPEVTCVVVDVSHEDPEVKFNWYVDGVEVHNAKTKPREEQYNSTYRVVSVLTVLHQDWLNGKEYKCKVSNKALPAPIEKTISKAKGQPREPQVYTLPPSRDELTKNQVSLTCLVKGFYPSDIAVEWESNGQPENNYKTTPPVLDSDGSFFLYSKLTVDKSRWQQGNVFSCSVMHEALHNHYTQKSLSLSPGK

SEQ ID NO: 11 - DNA, 855 bp, Artificial Sequence
  Nucleotides encoding Mouse TM4SF19(116-165)-Fc fusion protein
aaagatggtcccttttgcatgtttgatgtctcatccttcaatcagacacaagcttggaaattcggctatccctttaaagatctacacaacaggaattatctgtatgaccgttcactttggacctccgtttgcctggagccctctaaggctactagtgagcccaaatcttgtgacaaaactcacacatgcccaccgtgcccagcacctgaactcctggggggaccgtcagtcttcctcttccccccaaaacccaaggacaccctcatgatctcccggacccctgaggtcacatgcgtggtggtggacgtgagccacgaagaccctgaggtcaagttcaactggtacgtggacggcgtggaggtgcataatgccaagacaaagccgcgggaggagcagtacaacagcacgtaccgtgtggtcagcgtcctcaccgtcctgcaccaggactggctgaatggcaaggagtacaagtgcaaggtctccaacaaagccctcccagcccccatcgagaaaaccatctccaaagccaaagggcagccccgagaaccacaggtgtacaccctgcccccatcccgggatgagctgaccaagaaccaggtcagcctgacctgcctggtcaaaggcttctatcccagcgacatcgccgtggagtgggagagcaatgggcagccggagaacaactacaagaccacgcctcccgtgctggactccgacggctccttcttcctctacagcaagctcaccgtggacaagagcaggtggcagcaggggaacgtcttctcatgctccgtgatgcatgaggctctgcacaaccactacacgcagaagagcctctccctgtctccgggtaaatga

SEQ ID NO: 12 - protein, 50 aa, Homo sapiens
KDGPFCMFDVSSFNQTQAWKYGYPFKDLHSRNYLYDRSLWNSVCLEPSAA

SEQ ID NO: 13 - protein, 284 aa, Artificial Sequence
  Human TM4SF19(120-169)-Fc fusion protein
KDGPFCMFDVSSFNQTQAWKYGYPFKDLHSRNYLYDRSLWNSVCLEPSAATSEPKSCDKTHTCPPCPAPELLGGPSVFLFPPKPKDTLMISRTPEVTCVVVDVSHEDPEVKFNWYVDGVEVHNAKTKPREEQYNSTYRVVSVLTVLHQDWLNGKEYKCKVSNKALPAPIEKTISKAKGQPREPQVYTLPPSRDELTKNQVSLTCLVKGFYPSDIAVEWESNGQPENNYKTTPPVLDSDGSFFLYSKLTVDKSRWQQGNVFSCSVMHEALHNHYTQKSLSLSPGK

SEQ ID NO: 14 - DNA, 855 bp, Artificial Sequence
  Nucleotides encoding Human TM4SF19(120-169)-Fc fusion protein
aaagatggtcctttttgcatgtttgatgtttcatccttcaatcagacacaagcttggaaatatggttacccattcaaagacctgcatagtaggaattatctgtatgaccgttcgctctggaactccgtctgcctggagccctctgcagctactagtgagcccaaatcttgtgacaaaactcacacatgcccaccgtgcccagcacctgaactcctggggggaccgtcagtcttcctcttccccccaaaacccaaggacaccctcatgatctcccggacccctgaggtcacatgcgtggtggtggacgtgagccacgaagaccctgaggtcaagttcaactggtacgtggacggcgtggaggtgcataatgccaagacaaagccgcgggaggagcagtacaacagcacgtaccgtgtggtcagcgtcctcaccgtcctgcaccaggactggctgaatggcaaggagtacaagtgcaaggtctccaacaaagccctcccagcccccatcgagaaaaccatctccaaagccaaagggcagccccgagaaccacaggtgtacaccctgcccccatcccgggatgagctgaccaagaaccaggtcagcctgacctgcctggtcaaaggcttctatcccagcgacatcgccgtggagtgggagagcaatgggcagccggagaacaactacaagaccacgcctcccgtgctggactccgacggctccttcttcctctacagcaagctcaccgtggacaagagcaggtggcagcaggggaacgtcttctcatgctccgtgatgcatgaggctctgcacaaccactacacgcagaagagcctctccctgtctccgggtaaatga

SEQ ID NO: 15 - protein, 25 aa, Homo sapiens
KDLHSRNYLYDRSLWNSVCLEPSAA

SEQ ID NO: 16 - protein, 259 aa, Artificial Sequence
  Human TM4SF19(145-169)-Fc  fusion protein
KDLHSRNYLYDRSLWNSVCLEPSAATSEPKSCDKTHTCPPCPAPELLGGPSVFLFPPKPKDTLMISRTPEVTCVVVDVSHEDPEVKFNWYVDGVEVHNAKTKPREEQYNSTYRVVSVLTVLHQDWLNGKEYKCKVSNKALPAPIEKTISKAKGQPREPQVYTLPPSRDELTKNQVSLTCLVKGFYPSDIAVEWESNGQPENNYKTTPPVLDSDGSFFLYSKLTVDKSRWQQGNVFSCSVMHEALHNHYTQKSLSLSPGK

SEQ ID NO: 17 - DNA, 780 bp, Artificial Sequence
  Nucleotides encoding Human TM4SF19(145-169)-Fc  fusion protein
aaagacctgcatagtaggaattatctgtatgaccgttcgctctggaactccgtctgcctggagccctctgcagctactagtgagcccaaatcttgtgacaaaactcacacatgcccaccgtgcccagcacctgaactcctggggggaccgtcagtcttcctcttccccccaaaacccaaggacaccctcatgatctcccggacccctgaggtcacatgcgtggtggtggacgtgagccacgaagaccctgaggtcaagttcaactggtacgtggacggcgtggaggtgcataatgccaagacaaagccgcgggaggagcagtacaacagcacgtaccgtgtggtcagcgtcctcaccgtcctgcaccaggactggctgaatggcaaggagtacaagtgcaaggtctccaacaaagccctcccagcccccatcgagaaaaccatctccaaagccaaagggcagccccgagaaccacaggtgtacaccctgcccccatcccgggatgagctgaccaagaaccaggtcagcctgacctgcctggtcaaaggcttctatcccagcgacatcgccgtggagtgggagagcaatgggcagccggagaacaactacaagaccacgcctcccgtgctggactccgacggctccttcttcctctacagcaagctcaccgtggacaagagcaggtggcagcaggggaacgtcttctcatgctccgtgatgcatgaggctctgcacaaccactacacgcagaagagcctctccctgtctccgggtaaatga

SEQ ID NO: 18 - protein, 39 aa, Homo sapiens
SFNQTQAWKYGYPFKDLHSRNYLYDRSLWNSVCLEPSAA

SEQ ID NO: 19 - protein, 273 aa, Artificial Sequence
  Human TM4SF19(131-169)-Fc   fusion protein
SFNQTQAWKYGYPFKDLHSRNYLYDRSLWNSVCLEPSAATSEPKSCDKTHTCPPCPAPELLGGPSVFLFPPKPKDTLMISRTPEVTCVVVDVSHEDPEVKFNWYVDGVEVHNAKTKPREEQYNSTYRVVSVLTVLHQDWLNGKEYKCKVSNKALPAPIEKTISKAKGQPREPQVYTLPPSRDELTKNQVSLTCLVKGFYPSDIAVEWESNGQPENNYKTTPPVLDSDGSFFLYSKLTVDKSRWQQGNVFSCSVMHEALHNHYTQKSLSLSPGK

SEQ ID NO: 20 - DNA, 822 bp, Artificial Sequence
  Nucleotides encoding Human TM4SF19(131-169)-Fc   fusion protein
tccttcaatcagacacaagcttggaaatatggttacccattcaaagacctgcatagtaggaattatctgtatgaccgttcgctctggaactccgtctgcctggagccctctgcagctactagtgagcccaaatcttgtgacaaaactcacacatgcccaccgtgcccagcacctgaactcctggggggaccgtcagtcttcctcttccccccaaaacccaaggacaccctcatgatctcccggacccctgaggtcacatgcgtggtggtggacgtgagccacgaagaccctgaggtcaagttcaactggtacgtggacggcgtggaggtgcataatgccaagacaaagccgcgggaggagcagtacaacagcacgtaccgtgtggtcagcgtcctcaccgtcctgcaccaggactggctgaatggcaaggagtacaagtgcaaggtctccaacaaagccctcccagcccccatcgagaaaaccatctccaaagccaaagggcagccccgagaaccacaggtgtacaccctgcccccatcccgggatgagctgaccaagaaccaggtcagcctgacctgcctggtcaaaggcttctatcccagcgacatcgccgtggagtgggagagcaatgggcagccggagaacaactacaagaccacgcctcccgtgctggactccgacggctccttcttcctctacagcaagctcaccgtggacaagagcaggtggcagcaggggaacgtcttctcatgctccgtgatgcatgaggctctgcacaaccactacacgcagaagagcctctccctgtctccgggtaaatga

SEQ ID NO: 21 - protein, 61 aa, Homo sapiens
SGVALKDGPFCMFDVSSFNQTQAWKYGYPFKDLHSRNYLYDRSLWNSVCLEPSAAVVWHVS